European Patent Specification EP 4 136 457 B1, published February 19, 2025. Title: DETECTION ASSAYS FOR CORONAVIRUS NEUTRALIZING ANTIBODIES. Applicant: REGENERON PHARMACEUTICALS, INC. VYRIAD, INC. The sequence listing filed with the application follows.

SEQUENCE LISTING (75 sequences)

SEQ ID NO: 1 - protein, 1273 aa, Severe acute respiratory syndrome coronavirus 2
MFVFLVLLPLVSSQCVNLTTRTQLPPAYTNSFTRGVYYPDKVFRSSVLHSTQDLFLPFFSNVTWFHAIHVSGTNGTKRFDNPVLPFNDGVYFASTEKSNIIRGWIFGTTLDSKTQSLLIVNNATNVVIKVCEFQFCNDPFLGVYYHKNNKSWMESEFRVYSSANNCTFEYVSQPFLMDLEGKQGNFKNLREFVFKNIDGYFKIYSKHTPINLVRDLPQGFSALEPLVDLPIGINITRFQTLLALHRSYLTPGDSSSGWTAGAAAYYVGYLQPRTFLLKYNENGTITDAVDCALDPLSETKCTLKSFTVEKGIYQTSNFRVQPTESIVRFPNITNLCPFGEVFNATRFASVYAWNRKRISNCVADYSVLYNSASFSTFKCYGVSPTKLNDLCFTNVYADSFVIRGDEVRQIAPGQTGKIADYNYKLPDDFTGCVIAWNSNNLDSKVGGNYNYLYRLFRKSNLKPFERDISTEIYQAGSTPCNGVEGFNCYFPLQSYGFQPTNGVGYQPYRVVVLSFELLHAPATVCGPKKSTNLVKNKCVNFNFNGLTGTGVLTESNKKFLPFQQFGRDIADTTDAVRDPQTLEILDITPCSFGGVSVITPGTNTSNQVAVLYQDVNCTEVPVAIHADQLTPTWRVYSTGSNVFQTRAGCLIGAEHVNNSYECDIPIGAGICASYQTQTNSPRRARSVASQSIIAYTMSLGAENSVAYSNNSIAIPTNFTISVTTEILPVSMTKTSVDCTMYICGDSTECSNLLLQYGSFCTQLNRALTGIAVEQDKNTQEVFAQVKQIYKTPPIKDFGGFNFSQILPDPSKPSKRSFIEDLLFNKVTLADAGFIKQYGDCLGDIAARDLICAQKFNGLTVLPPLLTDEMIAQYTSALLAGTITSGWTFGAGAALQIPFAMQMAYRFNGIGVTQNVLYENQKLIANQFNSAIGKIQDSLSSTASALGKLQDVVNQNAQALNTLVKQLSSNFGAISSVLNDILSRLDKVEAEVQIDRLITGRLQSLQTYVTQQLIRAAEIRASANLAATKMSECVLGQSKRVDFCGKGYHLMSFPQSAPHGVVFLHVTYVPAQEKNFTTAPAICHDGKAHFPREGVFVSNGTHWFVTQRNFYEPQIITTDNTFVSGNCDVVIGIVNNTVYDPLQPELDSFKEELDKYFKNHTSPDVDLGDISGINASVVNIQKEIDRLNEVAKNLNESLIDLQELGKYEQYIKWPWYIWLGFIAGLIAIVMVTIMLCCMTSCCSCLKGCCSCGSCCKFDEDDSEPVLKGVKLHYT

SEQ ID NO: 2 - DNA, 3822 bp, Artificial Sequence
  source: /note="Description of Artificial Sequence: Synthetic polynucleotide"
atgttcgtcttcctggtcctgctgcctctggtctcctcacagtgcgtcaatctgacaactcggactcagctgccacctgcttatactaatagcttcaccagaggcgtgtactatcctgacaaggtgtttagaagctccgtgctgcactctacacaggatctgtttctgccattctttagcaacgtgacctggttccacgccatccacgtgagcggcaccaatggcacaaagcggttcgacaatcccgtgctgccttttaacgatggcgtgtacttcgcctctaccgagaagagcaacatcatcagaggctggatctttggcaccacactggactccaagacacagtctctgctgatcgtgaacaatgccaccaacgtggtcatcaaggtgtgcgagttccagttttgtaatgatcccttcctgggcgtgtactatcacaagaacaataagagctggatggagtccgagtttagagtgtattctagcgccaacaactgcacatttgagtacgtgagccagcctttcctgatggacctggagggcaagcagggcaatttcaagaacctgagggagttcgtgtttaagaatatcgacggctacttcaaaatctactctaagcacacccccatcaacctggtgcgcgacctgcctcagggcttcagcgccctggagcccctggtggatctgcctatcggcatcaacatcacccggtttcagacactgctggccctgcacagaagctacctgacacccggcgactcctctagcggatggaccgccggcgctgccgcctactatgtgggctacctccagccccggaccttcctgctgaagtacaacgagaatggcaccatcacagacgcagtggattgcgccctggaccccctgagcgagacaaagtgtacactgaagtcctttaccgtggagaagggcatctatcagacatccaatttcagggtgcagccaaccgagtctatcgtgcgctttcctaatatcacaaacctgtgcccatttggcgaggtgttcaacgcaacccgcttcgccagcgtgtacgcctggaataggaagcggatcagcaactgcgtggccgactatagcgtgctgtacaactccgcctctttcagcacctttaagtgctatggcgtgtcccccacaaagctgaatgacctgtgctttaccaacgtctacgccgattctttcgtgatcaggggcgacgaggtgcgccagatcgcccccggccagacaggcaagatcgcagactacaattataagctgccagacgatttcaccggctgcgtgatcgcctggaacagcaacaatctggattccaaagtgggcggcaactacaattatctgtaccggctgtttagaaagagcaatctgaagcccttcgagagggacatctctacagaaatctaccaggccggcagcaccccttgcaatggcgtggagggctttaactgttatttcccactccagtcctacggcttccagcccacaaacggcgtgggctatcagccttaccgcgtggtggtgctgagctttgagctgctgcacgccccagcaacagtgtgcggccccaagaagtccaccaatctggtgaagaacaagtgcgtgaacttcaacttcaacggcctgaccggcacaggcgtgctgaccgagtccaacaagaagttcctgccatttcagcagttcggcagggacatcgcagataccacagacgccgtgcgcgacccacagaccctggagatcctggacatcacaccctgctctttcggcggcgtgagcgtgatcacacccggcaccaatacaagcaaccaggtggccgtgctgtatcaggacgtgaattgtaccgaggtgcccgtggctatccacgccgatcagctgaccccaacatggcgggtgtacagcaccggctccaacgtcttccagacaagagccggatgcctgatcggagcagagcacgtgaacaattcctatgagtgcgacatcccaatcggcgccggcatctgtgcctcttaccagacccagacaaactctcccagaagagcccggagcgtggcctcccagtctatcatcgcctataccatgtccctgggcgccgagaacagcgtggcctactctaacaatagcatcgccatcccaaccaacttcacaatctctgtgaccacagagatcctgcccgtgtccatgaccaagacatctgtggactgcacaatgtatatctgtggcgattctaccgagtgcagcaacctgctgctccagtacggcagcttttgtacccagctgaatagagccctgacaggcatcgccgtggagcaggataagaacacacaggaggtgttcgcccaggtgaagcaaatctacaagaccccccctatcaaggactttggcggcttcaatttttcccagatcctgcctgatccatccaagccttctaagcggagctttatcgaggacctgctgttcaacaaggtgaccctggccgatgccggcttcatcaagcagtatggcgattgcctgggcgacatcgcagccagggacctgatctgcgcccagaagtttaatggcctgaccgtgctgccacccctgctgacagatgagatgatcgcacagtacacaagcgccctgctggccggcaccatcacatccggatggaccttcggcgcaggagccgccctccagatcccctttgccatgcagatggcctataggttcaacggcatcggcgtgacccagaatgtgctgtacgagaaccagaagctgatcgccaatcagtttaactccgccatcggcaagatccaggacagcctgtcctctacagccagcgccctgggcaagctccaggatgtggtgaatcagaacgcccaggccctgaataccctggtgaagcagctgagcagcaacttcggcgccatctctagcgtgctgaatgacatcctgagccggctggacaaggtggaggcagaggtgcagatcgaccggctgatcaccggccggctccagagcctccagacctatgtgacacagcagctgatcagggccgccgagatcagggccagcgccaatctggcagcaaccaagatgtccgagtgcgtgctgggccagtctaagagagtggacttttgtggcaagggctatcacctgatgtccttccctcagtctgccccacacggcgtggtgtttctgcacgtgacctacgtgcccgcccaggagaagaacttcaccacagcccctgccatctgccacgatggcaaggcccactttccaagggagggcgtgttcgtgtccaacggcacccactggtttgtgacacagcgcaatttctacgagccccagatcatcaccacagacaacaccttcgtgagcggcaactgtgacgtggtcatcggcatcgtgaacaataccgtgtatgatccactccagcccgagctggacagctttaaggaggagctggataagtatttcaagaatcacacctcccctgacgtggatctgggcgacatcagcggcatcaatgcctccgtggtgaacatccagaaggagatcgaccgcctgaacgaggtggctaagaatctgaacgagagcctgatcgacctccaggagctgggcaagtatgagcagtacatcaagtggccctggtacatctggctgggcttcatcgccggcctgatcgccatcgtgatggtgaccatcatgctgtgctgtatgacatcctgctgttcttgcctgaagggctgctgtagctgtggctcctgctgtaagtttgacgaggatgactctgaacctgtgctgaagggcgtgaagctgcattacacctaa

SEQ ID NO: 3 - protein, 1254 aa, Severe acute respiratory syndrome coronavirus 2
MFVFLVLLPLVSSQCVNLTTRTQLPPAYTNSFTRGVYYPDKVFRSSVLHSTQDLFLPFFSNVTWFHAIHVSGTNGTKRFDNPVLPFNDGVYFASTEKSNIIRGWIFGTTLDSKTQSLLIVNNATNVVIKVCEFQFCNDPFLGVYYHKNNKSWMESEFRVYSSANNCTFEYVSQPFLMDLEGKQGNFKNLREFVFKNIDGYFKIYSKHTPINLVRDLPQGFSALEPLVDLPIGINITRFQTLLALHRSYLTPGDSSSGWTAGAAAYYVGYLQPRTFLLKYNENGTITDAVDCALDPLSETKCTLKSFTVEKGIYQTSNFRVQPTESIVRFPNITNLCPFGEVFNATRFASVYAWNRKRISNCVADYSVLYNSASFSTFKCYGVSPTKLNDLCFTNVYADSFVIRGDEVRQIAPGQTGKIADYNYKLPDDFTGCVIAWNSNNLDSKVGGNYNYLYRLFRKSNLKPFERDISTEIYQAGSTPCNGVEGFNCYFPLQSYGFQPTNGVGYQPYRVVVLSFELLHAPATVCGPKKSTNLVKNKCVNFNFNGLTGTGVLTESNKKFLPFQQFGRDIADTTDAVRDPQTLEILDITPCSFGGVSVITPGTNTSNQVAVLYQDVNCTEVPVAIHADQLTPTWRVYSTGSNVFQTRAGCLIGAEHVNNSYECDIPIGAGICASYQTQTNSPRRARSVASQSIIAYTMSLGAENSVAYSNNSIAIPTNFTISVTTEILPVSMTKTSVDCTMYICGDSTECSNLLLQYGSFCTQLNRALTGIAVEQDKNTQEVFAQVKQIYKTPPIKDFGGFNFSQILPDPSKPSKRSFIEDLLFNKVTLADAGFIKQYGDCLGDIAARDLICAQKFNGLTVLPPLLTDEMIAQYTSALLAGTITSGWTFGAGAALQIPFAMQMAYRFNGIGVTQNVLYENQKLIANQFNSAIGKIQDSLSSTASALGKLQDVVNQNAQALNTLVKQLSSNFGAISSVLNDILSRLDKVEAEVQIDRLITGRLQSLQTYVTQQLIRAAEIRASANLAATKMSECVLGQSKRVDFCGKGYHLMSFPQSAPHGVVFLHVTYVPAQEKNFTTAPAICHDGKAHFPREGVFVSNGTHWFVTQRNFYEPQIITTDNTFVSGNCDVVIGIVNNTVYDPLQPELDSFKEELDKYFKNHTSPDVDLGDISGINASVVNIQKEIDRLNEVAKNLNESLIDLQELGKYEQYIKWPWYIWLGFIAGLIAIVMVTIMLCCMTSCCSCLKGCCSCGSCC

SEQ ID NO: 4 - DNA, 3765 bp, Artificial Sequence
  source: /note="Description of Artificial Sequence: Synthetic polynucleotide"
atgttcgtcttcctggtcctgctgcctctggtctcctcacagtgcgtcaatctgacaactcggactcagctgccacctgcttatactaatagcttcaccagaggcgtgtactatcctgacaaggtgtttagaagctccgtgctgcactctacacaggatctgtttctgccattctttagcaacgtgacctggttccacgccatccacgtgagcggcaccaatggcacaaagcggttcgacaatcccgtgctgccttttaacgatggcgtgtacttcgcctctaccgagaagagcaacatcatcagaggctggatctttggcaccacactggactccaagacacagtctctgctgatcgtgaacaatgccaccaacgtggtcatcaaggtgtgcgagttccagttttgtaatgatcccttcctgggcgtgtactatcacaagaacaataagagctggatggagtccgagtttagagtgtattctagcgccaacaactgcacatttgagtacgtgagccagcctttcctgatggacctggagggcaagcagggcaatttcaagaacctgagggagttcgtgtttaagaatatcgacggctacttcaaaatctactctaagcacacccccatcaacctggtgcgcgacctgcctcagggcttcagcgccctggagcccctggtggatctgcctatcggcatcaacatcacccggtttcagacactgctggccctgcacagaagctacctgacacccggcgactcctctagcggatggaccgccggcgctgccgcctactatgtgggctacctccagccccggaccttcctgctgaagtacaacgagaatggcaccatcacagacgcagtggattgcgccctggaccccctgagcgagacaaagtgtacactgaagtcctttaccgtggagaagggcatctatcagacatccaatttcagggtgcagccaaccgagtctatcgtgcgctttcctaatatcacaaacctgtgcccatttggcgaggtgttcaacgcaacccgcttcgccagcgtgtacgcctggaataggaagcggatcagcaactgcgtggccgactatagcgtgctgtacaactccgcctctttcagcacctttaagtgctatggcgtgtcccccacaaagctgaatgacctgtgctttaccaacgtctacgccgattctttcgtgatcaggggcgacgaggtgcgccagatcgcccccggccagacaggcaagatcgcagactacaattataagctgccagacgatttcaccggctgcgtgatcgcctggaacagcaacaatctggattccaaagtgggcggcaactacaattatctgtaccggctgtttagaaagagcaatctgaagcccttcgagagggacatctctacagaaatctaccaggccggcagcaccccttgcaatggcgtggagggctttaactgttatttcccactccagtcctacggcttccagcccacaaacggcgtgggctatcagccttaccgcgtggtggtgctgagctttgagctgctgcacgccccagcaacagtgtgcggccccaagaagtccaccaatctggtgaagaacaagtgcgtgaacttcaacttcaacggcctgaccggcacaggcgtgctgaccgagtccaacaagaagttcctgccatttcagcagttcggcagggacatcgcagataccacagacgccgtgcgcgacccacagaccctggagatcctggacatcacaccctgctctttcggcggcgtgagcgtgatcacacccggcaccaatacaagcaaccaggtggccgtgctgtatcaggacgtgaattgtaccgaggtgcccgtggctatccacgccgatcagctgaccccaacatggcgggtgtacagcaccggctccaacgtcttccagacaagagccggatgcctgatcggagcagagcacgtgaacaattcctatgagtgcgacatcccaatcggcgccggcatctgtgcctcttaccagacccagacaaactctcccagaagagcccggagcgtggcctcccagtctatcatcgcctataccatgtccctgggcgccgagaacagcgtggcctactctaacaatagcatcgccatcccaaccaacttcacaatctctgtgaccacagagatcctgcccgtgtccatgaccaagacatctgtggactgcacaatgtatatctgtggcgattctaccgagtgcagcaacctgctgctccagtacggcagcttttgtacccagctgaatagagccctgacaggcatcgccgtggagcaggataagaacacacaggaggtgttcgcccaggtgaagcaaatctacaagaccccccctatcaaggactttggcggcttcaatttttcccagatcctgcctgatccatccaagccttctaagcggagctttatcgaggacctgctgttcaacaaggtgaccctggccgatgccggcttcatcaagcagtatggcgattgcctgggcgacatcgcagccagggacctgatctgcgcccagaagtttaatggcctgaccgtgctgccacccctgctgacagatgagatgatcgcacagtacacaagcgccctgctggccggcaccatcacatccggatggaccttcggcgcaggagccgccctccagatcccctttgccatgcagatggcctataggttcaacggcatcggcgtgacccagaatgtgctgtacgagaaccagaagctgatcgccaatcagtttaactccgccatcggcaagatccaggacagcctgtcctctacagccagcgccctgggcaagctccaggatgtggtgaatcagaacgcccaggccctgaataccctggtgaagcagctgagcagcaacttcggcgccatctctagcgtgctgaatgacatcctgagccggctggacaaggtggaggcagaggtgcagatcgaccggctgatcaccggccggctccagagcctccagacctatgtgacacagcagctgatcagggccgccgagatcagggccagcgccaatctggcagcaaccaagatgtccgagtgcgtgctgggccagtctaagagagtggacttttgtggcaagggctatcacctgatgtccttccctcagtctgccccacacggcgtggtgtttctgcacgtgacctacgtgcccgcccaggagaagaacttcaccacagcccctgccatctgccacgatggcaaggcccactttccaagggagggcgtgttcgtgtccaacggcacccactggtttgtgacacagcgcaatttctacgagccccagatcatcaccacagacaacaccttcgtgagcggcaactgtgacgtggtcatcggcatcgtgaacaataccgtgtatgatccactccagcccgagctggacagctttaaggaggagctggataagtatttcaagaatcacacctcccctgacgtggatctgggcgacatcagcggcatcaatgcctccgtggtgaacatccagaaggagatcgaccgcctgaacgaggtggctaagaatctgaacgagagcctgatcgacctccaggagctgggcaagtatgagcagtacatcaagtggccctggtacatctggctgggcttcatcgccggcctgatcgccatcgtgatggtgaccatcatgctgtgctgtatgacatcctgctgttcttgcctgaagggctgctgtagctgtggctcctgctgttaa

SEQ ID NO: 5 - protein, 1258 aa, Artificial Sequence
  source: /note="Description of Artificial Sequence: Synthetic polypeptide"
MFVFLVLLPLVSSQCVNLTTRTQLPPAYTNSFTRGVYYPDKVFRSSVLHSTQDLFLPFFSNVTWFHAIHVSGTNGTKRFDNPVLPFNDGVYFASTEKSNIIRGWIFGTTLDSKTQSLLIVNNATNVVIKVCEFQFCNDPFLGVYYHKNNKSWMESEFRVYSSANNCTFEYVSQPFLMDLEGKQGNFKNLREFVFKNIDGYFKIYSKHTPINLVRDLPQGFSALEPLVDLPIGINITRFQTLLALHRSYLTPGDSSSGWTAGAAAYYVGYLQPRTFLLKYNENGTITDAVDCALDPLSETKCTLKSFTVEKGIYQTSNFRVQPTESIVRFPNITNLCPFGEVFNATRFASVYAWNRKRISNCVADYSVLYNSASFSTFKCYGVSPTKLNDLCFTNVYADSFVIRGDEVRQIAPGQTGKIADYNYKLPDDFTGCVIAWNSNNLDSKVGGNYNYLYRLFRKSNLKPFERDISTEIYQAGSTPCNGVEGFNCYFPLQSYGFQPTNGVGYQPYRVVVLSFELLHAPATVCGPKKSTNLVKNKCVNFNFNGLTGTGVLTESNKKFLPFQQFGRDIADTTDAVRDPQTLEILDITPCSFGGVSVITPGTNTSNQVAVLYQDVNCTEVPVAIHADQLTPTWRVYSTGSNVFQTRAGCLIGAEHVNNSYECDIPIGAGICASYQTQTNSPRRARSVASQSIIAYTMSLGAENSVAYSNNSIAIPTNFTISVTTEILPVSMTKTSVDCTMYICGDSTECSNLLLQYGSFCTQLNRALTGIAVEQDKNTQEVFAQVKQIYKTPPIKDFGGFNFSQILPDPSKPSKRSFIEDLLFNKVTLADAGFIKQYGDCLGDIAARDLICAQKFNGLTVLPPLLTDEMIAQYTSALLAGTITSGWTFGAGAALQIPFAMQMAYRFNGIGVTQNVLYENQKLIANQFNSAIGKIQDSLSSTASALGKLQDVVNQNAQALNTLVKQLSSNFGAISSVLNDILSRLDKVEAEVQIDRLITGRLQSLQTYVTQQLIRAAEIRASANLAATKMSECVLGQSKRVDFCGKGYHLMSFPQSAPHGVVFLHVTYVPAQEKNFTTAPAICHDGKAHFPREGVFVSNGTHWFVTQRNFYEPQIITTDNTFVSGNCDVVIGIVNNTVYDPLQPELDSFKEELDKYFKNHTSPDVDLGDISGINASVVNIQKEIDRLNEVAKNLNESLIDLQELGKYEQYIKWPWYIWLGFIAGLIAIVMVTIMLCCMKLKHTKKRQIYTDIEMNRLGK

SEQ ID NO: 6 - DNA, 3777 bp, Artificial Sequence
  source: /note="Description of Artificial Sequence: Synthetic polynucleotide"
atgttcgtcttcctggtcctgctgcctctggtctcctcacagtgcgtcaatctgacaactcggactcagctgccacctgcttatactaatagcttcaccagaggcgtgtactatcctgacaaggtgtttagaagctccgtgctgcactctacacaggatctgtttctgccattctttagcaacgtgacctggttccacgccatccacgtgagcggcaccaatggcacaaagcggttcgacaatcccgtgctgccttttaacgatggcgtgtacttcgcctctaccgagaagagcaacatcatcagaggctggatctttggcaccacactggactccaagacacagtctctgctgatcgtgaacaatgccaccaacgtggtcatcaaggtgtgcgagttccagttttgtaatgatcccttcctgggcgtgtactatcacaagaacaataagagctggatggagtccgagtttagagtgtattctagcgccaacaactgcacatttgagtacgtgagccagcctttcctgatggacctggagggcaagcagggcaatttcaagaacctgagggagttcgtgtttaagaatatcgacggctacttcaaaatctactctaagcacacccccatcaacctggtgcgcgacctgcctcagggcttcagcgccctggagcccctggtggatctgcctatcggcatcaacatcacccggtttcagacactgctggccctgcacagaagctacctgacacccggcgactcctctagcggatggaccgccggcgctgccgcctactatgtgggctacctccagccccggaccttcctgctgaagtacaacgagaatggcaccatcacagacgcagtggattgcgccctggaccccctgagcgagacaaagtgtacactgaagtcctttaccgtggagaagggcatctatcagacatccaatttcagggtgcagccaaccgagtctatcgtgcgctttcctaatatcacaaacctgtgcccatttggcgaggtgttcaacgcaacccgcttcgccagcgtgtacgcctggaataggaagcggatcagcaactgcgtggccgactatagcgtgctgtacaactccgcctctttcagcacctttaagtgctatggcgtgtcccccacaaagctgaatgacctgtgctttaccaacgtctacgccgattctttcgtgatcaggggcgacgaggtgcgccagatcgcccccggccagacaggcaagatcgcagactacaattataagctgccagacgatttcaccggctgcgtgatcgcctggaacagcaacaatctggattccaaagtgggcggcaactacaattatctgtaccggctgtttagaaagagcaatctgaagcccttcgagagggacatctctacagaaatctaccaggccggcagcaccccttgcaatggcgtggagggctttaactgttatttcccactccagtcctacggcttccagcccacaaacggcgtgggctatcagccttaccgcgtggtggtgctgagctttgagctgctgcacgccccagcaacagtgtgcggccccaagaagtccaccaatctggtgaagaacaagtgcgtgaacttcaacttcaacggcctgaccggcacaggcgtgctgaccgagtccaacaagaagttcctgccatttcagcagttcggcagggacatcgcagataccacagacgccgtgcgcgacccacagaccctggagatcctggacatcacaccctgctctttcggcggcgtgagcgtgatcacacccggcaccaatacaagcaaccaggtggccgtgctgtatcaggacgtgaattgtaccgaggtgcccgtggctatccacgccgatcagctgaccccaacatggcgggtgtacagcaccggctccaacgtcttccagacaagagccggatgcctgatcggagcagagcacgtgaacaattcctatgagtgcgacatcccaatcggcgccggcatctgtgcctcttaccagacccagacaaactctcccagaagagcccggagcgtggcctcccagtctatcatcgcctataccatgtccctgggcgccgagaacagcgtggcctactctaacaatagcatcgccatcccaaccaacttcacaatctctgtgaccacagagatcctgcccgtgtccatgaccaagacatctgtggactgcacaatgtatatctgtggcgattctaccgagtgcagcaacctgctgctccagtacggcagcttttgtacccagctgaatagagccctgacaggcatcgccgtggagcaggataagaacacacaggaggtgttcgcccaggtgaagcaaatctacaagaccccccctatcaaggactttggcggcttcaatttttcccagatcctgcctgatccatccaagccttctaagcggagctttatcgaggacctgctgttcaacaaggtgaccctggccgatgccggcttcatcaagcagtatggcgattgcctgggcgacatcgcagccagggacctgatctgcgcccagaagtttaatggcctgaccgtgctgccacccctgctgacagatgagatgatcgcacagtacacaagcgccctgctggccggcaccatcacatccggatggaccttcggcgcaggagccgccctccagatcccctttgccatgcagatggcctataggttcaacggcatcggcgtgacccagaatgtgctgtacgagaaccagaagctgatcgccaatcagtttaactccgccatcggcaagatccaggacagcctgtcctctacagccagcgccctgggcaagctccaggatgtggtgaatcagaacgcccaggccctgaataccctggtgaagcagctgagcagcaacttcggcgccatctctagcgtgctgaatgacatcctgagccggctggacaaggtggaggcagaggtgcagatcgaccggctgatcaccggccggctccagagcctccagacctatgtgacacagcagctgatcagggccgccgagatcagggccagcgccaatctggcagcaaccaagatgtccgagtgcgtgctgggccagtctaagagagtggacttttgtggcaagggctatcacctgatgtccttccctcagtctgccccacacggcgtggtgtttctgcacgtgacctacgtgcccgcccaggagaagaacttcaccacagcccctgccatctgccacgatggcaaggcccactttccaagggagggcgtgttcgtgtccaacggcacccactggtttgtgacacagcgcaatttctacgagccccagatcatcaccacagacaacaccttcgtgagcggcaactgtgacgtggtcatcggcatcgtgaacaataccgtgtatgatccactccagcccgagctggacagctttaaggaggagctggataagtatttcaagaatcacacctcccctgacgtggatctgggcgacatcagcggcatcaatgcctccgtggtgaacatccagaaggagatcgaccgcctgaacgaggtggctaagaatctgaacgagagcctgatcgacctccaggagctgggcaagtatgagcagtacatcaagtggccctggtacatctggctgggcttcatcgccggcctgatcgccatcgtgatggtgaccatcatgctgtgctgtatgaaattaaagcacaccaagaaaagacagatttatacagacatagagatgaaccgacttggaaagtaa

SEQ ID NO: 7 - protein, 237 aa, Artificial Sequence
  source: /note="Description of Artificial Sequence: Synthetic polypeptide"
MSSLKKILGLKGKGKKSKKLGIAPPPYEEDTSMEYAPSAPIDKSYFGVDERDTHDPNQLRYEKSFFTVKMTVRSNRPFRTYSDVAAAVSHWDHMYIGMAGKRPFYKILAFLGSSNLKATPAVLADQGQPEYHAHCEGRAYLPHRMGKTPPMLNVPEHFRRPFNIGLYKGTIELTMTIYDDESLEAAPMIWDHFNSSKFSDFREKALMFGLIVEEEASGAWVLDSVRHSKWASLASSF

SEQ ID NO: 8 - DNA, 690 bp, Artificial Sequence
  source: /note="Description of Artificial Sequence: Synthetic polynucleotide"
atgagttccttaaagaagattctcggtctgaaggggaaaggtaagaaatctaagaaattagggatcgcaccacccccttatgaagaggacactagcatggagtatgctccgagcgctccaattgacaaatcctattttggagttgacgagcgagacacctatgatccgaatcaattaagatatgagaaattcttctttacagtgaaaatgacggttagatctaatcgtccgttcagaacatactcagatgtggcagccgctgtatcccattgggatcacatgtacatcggaatggcagggaaacgtcccttctacaaaatcttggcttttttgggttcttctaatctaaaggccactccagcggtattggcagatcaaggtcaaccagagtatcacgctcactgcgaaggcagggcttatttgccacataggatggggaagacccctcccatgctcaatgtaccagagcacttcagaagaccattcaatataggtctttacaagggaacgattgagctcacaatgaccatctacgatgatgagtcactggaagcagctcctatgatctgggatcatttcaattcttccaaattttctgatttcagagagaaggccttaatgtttggcctgattgtcgagaaaaaggcatctggagcgtgggtcctggactctatcggccacttcaaatga

SEQ ID NO: 9 - protein, 237 aa, Vesicular stomatitis virus
MSSLKKILGLKGKGKKSKKLGIAPPPYEEDTSMEYAPSAPIDKSYFGVDEMDTHDPNQLRYEKSFFTVKMTVRSNRPFRTYSDVAAAVSHWDHMYIGMAGKRPFYKILAFLGSSNLKATPAVLADQGQPEYHAHCEGRAYLPHRMGKTPPMLNVPEHFRRPFNIGLYKGTIELTMTIYDDESLEAAPMIWDHFNSSKFSDFREKALMFGLIVEEEASGAWVLDSVRHSKWASLASSF

SEQ ID NO: 10 - DNA, 690 bp, Vesicular stomatitis virus
atgagttccttaaagaagattctcggtctgaaggggaaaggtaagaaatctaagaaattagggatcgcaccacccccttatgaagaggacactagcatggagtatgctccgagcgctccaattgacaaatcctattttggagttgacgagatggacacctatgatccgaatcaattaagatatgagaaattcttctttacagtgaaaatgacggttagatctaatcgtccgttcagaacatactcagatgtggcagccgctgtatcccattgggatcacatgtacatcggaatggcagggaaacgtcccttctacaaaatcttggcttttttgggttcttctaatctaaaggccactccagcggtattggcagatcaaggtcaaccagagtatcacgctcactgcgaaggcagggcttatttgccacataggatggggaagacccctcccatgctcaatgtaccagagcacttcagaagaccattcaatataggtctttacaagggaacgattgagctcacaatgaccatctacgatgatgagtcactggaagcagctcctatgatctgggatcatttcaattcttccaaattttctgatttcagagagaaggccttaatgtttggcctgattgtcgagaaaaaggcatctggagcgtgggtcctggactctatcggccacttcaaatga

SEQ ID NO: 11 - DNA, 7 bp, Vesicular stomatitis virus
cactatg

SEQ ID NO: 12 - DNA, 7 bp, Artificial Sequence
  source: /note="Description of Artificial Sequence: Synthetic oligonucleotide"
caccatg

SEQ ID NO: 13 - protein, 1185 aa, Severe acute respiratory syndrome coronavirus
MFIFLLFLTLTSGSDLDRCTTFDDVQAPNYTQHTSSMRGVYYPDEIFRSDTLYLTQDLFLPFYSNVTGFHTINHTFGNPVIPFKDGIYFAATEKSNVVRGWVFGSTMNNKSQSVIIINNSTNVVIRACNFELCDNPFFAVSKPMGTQTHTMIFDNAFNCTFEYISDAFSLDVSEKSGNFKHLREFVFKNKDGFLYVYKGYQPIDVVRDLPSGFNTLKPIFKLPLGINITNFRAILTAFSPAQDIWGTSAAAYFVGYLKPTTFMLKYDENGTITDAVDCSQNPLAELKCSVKSFEIDKGIYQTSNFRVVPSGDVVRFPNITNLCPFGEVFNATKFPSVYAWERKKISNCVADYSVLYNSTFFSTFKCYGVSATKLNDLCFSNVYADSFVVKGDDVRQIAPGQTGVIADYNYKLPDDFMGCVLAWNTRNIDATSTGNYNYKYRYLRHGKLRPFERDISNVPFSPDGKPCTPPALNCYWPLNDYGFYTTTGIGYQPYRVVVLSFELLNAPATVCGPKLSTDLIKNQCVNFNFNGLTGTGVLTPSSKRFQPFQQFGRDVSDFTDSVRDPKTSEILDISPCSFGGVSVITPGTNASSEVAVLYQDVNCTDVSTAIHADQLTPAWRIYSTGNNVNFSISITTEVMPVSMAKTSVDCNMYICGDSTECANLLLQYGSFCTQLNRALSGIAAEQDRNTREVFAQVKQMYKTPTLKYFGGFNFSQILPDPLKPTKRSFIEDLLFNKVTLADAGFMKQYGECLGDINARDLICAQKFNGLTVLPPLLTDDMIAAYTAALVSGTATAGWTFGAGAALQIPFAMQMAYRFNGIGVTQNVLYENQKQIANQFNKAISQIQESLTTTSTALGKLQDVVNQNAQALNTLVKQLSSNFGAISSVLNDILSRLDKVEAEVQIDRLITGRLQSLQTYVTQQLIRAAEIRASANLAATKMSECVLGQSKRVDFCGKGYHLMSFPQAAPHGVVFLHVTYVPSQERNFTTAPAICHEGKAYFPREGVFVFNGTSWFITQRNFFSPQIITTDNTFVSGNCDVVIGIINNTVYDPLQPELDSFKEELDKYFKNHTSPDVDLGDISGINASVVNIQKEIDRLNEVAKNLNESLIDLQELGKYEQYIKWPWYVWLGFIAGLIAIVMVTILLCCMTSCCSCLKGACSCGSCCKFDEDDSEPVLKGVKLHYT

SEQ ID NO: 14 - protein, 316 aa, Artificial Sequence
  source: /note="Description of Artificial Sequence: Synthetic polypeptide"
MASKVYDPEQRKRMITGPQWWARCKQMNVLDSFINYYDSEKHAENAVIFLHGNATSSYLWRHVVPHIEPVARCIIPDLIGMGKSGKSGNGSYRLLDHYKYLTAWFELLNLPKKIIFVGHDWGAALAFHYAYEHQDRIKAIVHMESVVDVIESWDESGGGGMSKGEELFTGVVPILVELDGDVNGHKFSVRGEGEGDATIGKLTLKFICTTGKLPVPWPTLVTTLTYGVQCFSRYPDHMKRHDFFKSAMPEGYVQERTISFKDDGKYKTRAVVKFEGDTLVNRIELKGTDFKEDGNILGHKLEYNFNSHNVYITADK

SEQ ID NO: 15 - DNA, 4093 bp, Artificial Sequence
  source: /note="Description of Artificial Sequence: Synthetic polynucleotide"
agatcttcaatattggccattagccatattattcattggttatatagcataaatcaatattggctattggccattgcatacgttgtatctatatcataatatgtacatttatattggctcatgtccaatatgaccgccatgttggcattgattattgactagttattaatagtaatcaattacggggtcattagttcatagcccatatatggagttccgcgttacataacttacggtaaatggcccgcctggctgaccgcccaacgacccccgcccattgacgtcaataatgacgtatgttcccatagtaacgccaatagggactttccattgacgtcaatgggtggagtatttacggtaaactgcccacttggcagtacatcaagtgtatcatatgccaagtccgccccctattgacgtcaatgacggtaaatggcccgcctggcattatgcccagtacatgaccttacgggactttcctacttggcagtacatctacgtattagtcatcgctattaccatggtgatgcggttttggcagtacaccaatgggcgtggatagcggtttgactcacggggatttccaagtctccaccccattgacgtcaatgggagtttgttttggcaccaaaatcaacgggactttccaaaatgtcgtaataaccccgccccgttgacgcaaatgggcggtaggcgtgtacggtgggaggtctatataagcagagctcgtttagtgaaccgtcagatcactagaagctttattgcggtagtttatcacagttaaattgctaacgcagtcagtgcttctgacacaacagtctcgaacttaagctgcagaagttggtcgtgaggcactgggcaggtaagtatcaaggttacaagacaggtttaaggagaccaatagaaactgggcttgtcgagacagagaagactcttgcgtttctgataggcacctattggtcttactgacatccactttgcctttctctccacaggtgtccactcccagttcaattacagctcttaaggctagagtacttaatacgactcactataggctagccaccatggcttccaaggtgtacgaccccgagcaacgcaaacgcatgatcactgggcctcagtggtgggctcgctgcaagcaaatgaacgtgctggactccttcatcaactactatgattccgagaagcacgccgagaacgccgtgatttttctgcatggtaacgctacctccagctacctgtggaggcacgtcgtgcctcacatcgagcccgtggctagatgcatcatccctgatctgatcggaatgggtaagtccggcaagagcgggaatggctcatatcgcctcctggatcactacaagtacctcaccgcttggttcgagctgctgaaccttccaaagaaaatcatctttgtgggccacgactggggggctgctctggcctttcactacgcctacgagcaccaagacaggatcaaggccatcgtccatatggagagtgtcgtggacgtgatcgagtcctgggacgagtccggaggaggcggaatgagcaagggcgaggagctgttcaccggcgtggtgcccatcctggtggagctggacggcgacgtgaacggccacaagttcagcgtgagaggcgagggcgagggcgacgccaccatcggcaagctgaccctgaagttcatctgcaccaccggcaagctgcccgtgccctggcccaccctggtgaccaccctgacctacggcgtgcagtgcttcagcagataccccgaccacatgaagagacacgacttcttcaagagcgccatgcccgagggctacgtgcaggagagaaccatcagcttcaaggacgacggcaagtacaagaccagagccgtggtgaagttcgagggcgacaccctggtgaacagaatcgagctgaagggcaccgacttcaaggaggacggcaacatcctgggccacaagctggagtacaacttcaacagccacaacgtgtacatcaccgccgacaagtgatctagagcggccgcttcgagcagacatgataagatacattgatgagtttggacaaaccacaactagaatgcagtgaaaaaaatgctttatttgtgaaatttgtgatgctattgctttatttgtaaccattataagctgcaataaacaagttaacaacaacaattgcattcattttatgtttcaggttcagggggaggtgtgggaggttttttaaagcaagtaaaacctctacaaatgtggtaaaatcgataaggatccaggtggcacttttcggggaaatgtgcgcggaacccctatttgtttatttttctaaatacattcaaatatgtatccgctcatgagacaataaccctgataaatgcttcaataatattgaaaaaggaagagtatgagtattcaacatttccgtgtcgcccttattcccttttttgcggcattttgccttcctgtttttgctcacccagaaacgctggtgaaagtaaaagatgctgaagatcagttgggtgcacgagtgggttacatcgaactggatctcaacagcggtaagatccttgagagttttcgccccgaagaacgttttccaatgatgagcacttttaaagttctgctatgtggcgcggtattatcccgtattgacgccgggcaagagcaactcggtcgccgcatacactattctcagaatgacttggttgagtactcaccagtcacagaaaagcatcttacggatggcatgacagtaagagaattatgcagtgctgccataaccatgagtgataacactgcggccaacttacttctgacaacgatcggaggaccgaaggagctaaccgcttttttgcacaacatgggggatcatgtaactcgccttgatcgttgggaaccggagctgaatgaagccataccaaacgacgagcgtgacaccacgatgcctgtagcaatggcaacaacgttgcgcaaactattaactggcgaactacttactctagcttcccggcaacaattaatagactggatggaggcggataaagttgcaggaccacttctgcgctcggcccttccggctggctggtttattgctgataaatctggagccggtgagcgtgggtctcgcggtatcattgcagcactggggccagatggtaagccctcccgtatcgtagttatctacacgacggggagtcaggcaactatggatgaacgaaatagacagatcgctgagataggtgcctcactgattaagcattggtaactgtcagaccaagtttactcatatatactttagattgatttaaaacttcatttttaatttaaaaggatctaggtgaagatcctttttgataatctcatgaccaaaatcccttaacgtgagttttcgttccactgagcgtcagaccccgtagaaaagatcaaaggatcttcttgagatcctttttttctgcgcgtaatctgctgcttgcaaacaaaaaaaccaccgctaccagcggtggtttgtttgccggatcaagagctaccaactctttttccgaaggtaactggcttcagcagagcgcagataccaaatactgttcttctagtgtagccgtagttaggccaccacttcaagaactctgtagcaccgcctacatacctcgctctgctaatcctgttaccagtggctgctgccagtggcgataagtcgtgtcttaccgggttggactcaagacgatagttaccggataaggcgcagcggtcgggctgaacggggggttcgtgcacacagcccagcttggagcgaacgacctacaccgaactgagatacctacagcgtgagctatgagaaagcgccacgcttcccgaagggagaaaggcggacaggtatccggtaagcggcagggtcggaacaggagagcgcacgagggagcttccagggggaaacgcctggtatctttatagtcctgtcgggtttcgccacctctgacttgagcgtcgatttttgtgatgctcgtcaggggggcggagcctatggaaaaacgccagcaacgcggcctttttacggttcctggccttttgctggccttttgctcacatggctcgac

SEQ ID NO: 16 - protein, 236 aa, Artificial Sequence
  source: /note="Description of Artificial Sequence: Synthetic polypeptide"
MQKNGIKANFTVRHNVEDGSVQLADHYQQNTPIGDGPVLLPDNHYLSTQTVLSKDPNEKRDHMVLHEYVNAAGITGGGGSWPDIEEDIALIKSEEGEKMVLENNFFVETVLPSKIMRKLEPEEFAAYLEPFKEKGEVRRPTLSWPREIPLVKGGKPDVVQIVRNYNAYLRASDDLPKLFIESDPGFFSNAIVEGAKKFPNTEFVKVKGLHFLQEDAPDEMGKYIKSFVERVLKNEQ

SEQ ID NO: 17 - DNA, 3854 bp, Artificial Sequence
  source: /note="Description of Artificial Sequence: Synthetic polynucleotide"
agatcttcaatattggccattagccatattattcattggttatatagcataaatcaatattggctattggccattgcatacgttgtatctatatcataatatgtacatttatattggctcatgtccaatatgaccgccatgttggcattgattattgactagttattaatagtaatcaattacggggtcattagttcatagcccatatatggagttccgcgttacataacttacggtaaatggcccgcctggctgaccgcccaacgacccccgcccattgacgtcaataatgacgtatgttcccatagtaacgccaatagggactttccattgacgtcaatgggtggagtatttacggtaaactgcccacttggcagtacatcaagtgtatcatatgccaagtccgccccctattgacgtcaatgacggtaaatggcccgcctggcattatgcccagtacatgaccttacgggactttcctacttggcagtacatctacgtattagtcatcgctattaccatggtgatgcggttttggcagtacaccaatgggcgtggatagcggtttgactcacggggatttccaagtctccaccccattgacgtcaatgggagtttgttttggcaccaaaatcaacgggactttccaaaatgtcgtaataaccccgccccgttgacgcaaatgggcggtaggcgtgtacggtgggaggtctatataagcagagctcgtttagtgaaccgtcagatcactagaagctttattgcggtagtttatcacagttaaattgctaacgcagtcagtgcttctgacacaacagtctcgaacttaagctgcagaagttggtcgtgaggcactgggcaggtaagtatcaaggttacaagacaggtttaaggagaccaatagaaactgggcttgtcgagacagagaagactcttgcgtttctgataggcacctattggtcttactgacatccactttgcctttctctccacaggtgtccactcccagttcaattacagctcttaaggctagagtacttaatacgactcactataggctagccaccatgcagaagaacggcatcaaggccaacttcaccgtgagacacaacgtggaggacggcagcgtgcagctggccgaccactaccagcagaacacccccatcggcgacggccccgtgctgctgcccgacaaccactacctgagcacccagaccgtgctgagcaaggaccccaacgagaagagagaccacatggtgctgcacgagtacgtgaacgccgccggcatcaccggcggtggcggatcctggcctgacatcgaggaggatatcgccctgatcaagagcgaagagggcgagaaaatggtgcttgagaataacttcttcgtcgagaccgtgctcccaagcaagatcatgcggaaactggagcctgaggagttcgctgcctacctggagccattcaaggagaagggcgaggttagacggcctaccctctcctggcctcgcgagatccctctcgttaagggaggcaagcccgacgtcgtccagattgtccgcaactacaacgcctaccttcgggccagcgacgatctgcctaagctgttcatcgagtccgaccctgggttcttttccaacgctattgtcgagggagctaagaagttccctaacaccgagttcgtgaaggtgaagggcctccacttcctccaggaggacgctccagatgaaatgggtaagtacatcaagagcttcgtggagcgcgtgctgaagaacgagcagtaattctagagcggccgcttcgagcagacatgataagatacattgatgagtttggacaaaccacaactagaatgcagtgaaaaaaatgctttatttgtgaaatttgtgatgctattgctttatttgtaaccattataagctgcaataaacaagttaacaacaacaattgcattcattttatgtttcaggttcagggggaggtgtgggaggttttttaaagcaagtaaaacctctacaaatgtggtaaaatcgataaggatccaggtggcacttttcggggaaatgtgcgcggaacccctatttgtttatttttctaaatacattcaaatatgtatccgctcatgagacaataaccctgataaatgcttcaataatattgaaaaaggaagagtatgagtattcaacatttccgtgtcgcccttattcccttttttgcggcattttgccttcctgtttttgctcacccagaaacgctggtgaaagtaaaagatgctgaagatcagttgggtgcacgagtgggttacatcgaactggatctcaacagcggtaagatccttgagagttttcgccccgaagaacgttttccaatgatgagcacttttaaagttctgctatgtggcgcggtattatcccgtattgacgccgggcaagagcaactcggtcgccgcatacactattctcagaatgacttggttgagtactcaccagtcacagaaaagcatcttacggatggcatgacagtaagagaattatgcagtgctgccataaccatgagtgataacactgcggccaacttacttctgacaacgatcggaggaccgaaggagctaaccgcttttttgcacaacatgggggatcatgtaactcgccttgatcgttgggaaccggagctgaatgaagccataccaaacgacgagcgtgacaccacgatgcctgtagcaatggcaacaacgttgcgcaaactattaactggcgaactacttactctagcttcccggcaacaattaatagactggatggaggcggataaagttgcaggaccacttctgcgctcggcccttccggctggctggtttattgctgataaatctggagccggtgagcgtgggtctcgcggtatcattgcagcactggggccagatggtaagccctcccgtatcgtagttatctacacgacggggagtcaggcaactatggatgaacgaaatagacagatcgctgagataggtgcctcactgattaagcattggtaactgtcagaccaagtttactcatatatactttagattgatttaaaacttcatttttaatttaaaaggatctaggtgaagatcctttttgataatctcatgaccaaaatcccttaacgtgagttttcgttccactgagcgtcagaccccgtagaaaagatcaaaggatcttcttgagatcctttttttctgcgcgtaatctgctgcttgcaaacaaaaaaaccaccgctaccagcggtggtttgtttgccggatcaagagctaccaactctttttccgaaggtaactggcttcagcagagcgcagataccaaatactgttcttctagtgtagccgtagttaggccaccacttcaagaactctgtagcaccgcctacatacctcgctctgctaatcctgttaccagtggctgctgccagtggcgataagtcgtgtcttaccgggttggactcaagacgatagttaccggataaggcgcagcggtcgggctgaacggggggttcgtgcacacagcccagcttggagcgaacgacctacaccgaactgagatacctacagcgtgagctatgagaaagcgccacgcttcccgaagggagaaaggcggacaggtatccggtaagcggcagggtcggaacaggagagcgcacgagggagcttccagggggaaacgcctggtatctttatagtcctgtcgggtttcgccacctctgacttgagcgtcgatttttgtgatgctcgtcaggggggcggagcctatggaaaaacgccagcaacgcggcctttttacggttcctggccttttgctggccttttgctcacatggctcgac

SEQ ID NO: 18 - protein, 231 aa, Artificial Sequence
  source: /note="Description of Artificial Sequence: Synthetic polypeptide"
MSKGEELFTGVVPILVELDGDVNGHKFSVRGEGEGDATIGKLTLKFICTTGKLPVPWPTLVTTLTYGVQCFSRYPDHMKRHDFFKSAMPEGYVQERTISFKDDGKYKTRAVVKFEGDTLVNRIELKGTDFKEDGNILGHKLEYNFNSHNVYITADKMQKNGIKANFTVRHNVEDGSVQLADHYQQNTPIGDGPVLLPDNHYLSTQTVLSKDPNEKRDHMVLHEYVNAAGIT

SEQ ID NO: 19 - protein, 311 aa, Artificial Sequence
  source: /note="Description of Artificial Sequence: Synthetic polypeptide"
MASKVYDPEQRKRMITGPQWWARCKQMNVLDSFINYYDSEKHAENAVIFLHGNATSSYLWRHVVPHIEPVARCIIPDLIGMGKSGKSGNGSYRLLDHYKYLTAWFELLNLPKKIIFVGHDWGAALAFHYAYEHQDRIKAIVHMESVVDVIESWDEWPDIEEDIALIKSEEGEKMVLENNFFVETVLPSKIMRKLEPEEFAAYLEPFKEKGEVRRPTLSWPREIPLVKGGKPDVVQIVRNYNAYLRASDDLPKLFIESDPGFFSNAIVEGAKKFPNTEFVKVKGLHFLQEDAPDEMGKYIKSFVERVLKNEQ

SEQ ID NO: 20 - protein, 19 aa, Severe acute respiratory syndrome coronavirus 2
KFDEDDSEPVLKGVKLHYT

SEQ ID NO: 21 - protein, 21 aa, Vesicular stomatitis virus
KLKHTKKRQIYTDIEMNRLGK

SEQ ID NO: 22 - protein, 117 aa, Artificial Sequence
  source: /note="Description of Artificial Sequence: Synthetic polypeptide"
EVQLVESGGGLVQPGGSLRLSCAASGLIVSRNYMIWVRQAPGKGLEWVSVIYSGGSTFYADSVKGRFTISRHNSKNTLYLQMNSLRAEDTAVYYCARDLGTGGMDVWGQGTTVTVSS

SEQ ID NO: 23 - DNA, 351 bp, Artificial Sequence
  source: /note="Description of Artificial Sequence: Synthetic polynucleotide"
gaggtgcagctggtggagtctggaggaggcttggtccagcctggggggtccctgagactctcctgtgcagcctctgggttaatagtcagtcgcaactacatgatctgggtccgccaggctccagggaaggggctggagtgggtctcagttatttatagcggtggtagcacattctacgcagactccgtgaagggccgattcaccatctccagacacaattccaagaacacgctgtatcttcaaatgaacagcctgagggctgaggacacggccgtatattactgtgcgagagatctgggtacaggaggtatggacgtctggggccaagggaccacggtcaccgtctcctca

SEQ ID NO: 24 - protein, 8 aa, Artificial Sequence
  source: /note="Description of Artificial Sequence: Synthetic peptide"
GLIVSRNY

SEQ ID NO: 25 - DNA, 24 bp, Artificial Sequence
  source: /note="Description of Artificial Sequence: Synthetic oligonucleotide"
gggttaatagtcagtcgcaactac

SEQ ID NO: 26 - protein, 7 aa, Artificial Sequence
  source: /note="Description of Artificial Sequence: Synthetic peptide"
IYSGGST

SEQ ID NO: 27 - DNA, 21 bp, Artificial Sequence
  source: /note="Description of Artificial Sequence: Synthetic oligonucleotide"
atttatagcggtggtagcaca

SEQ ID NO: 28 - protein, 11 aa, Artificial Sequence
  source: /note="Description of Artificial Sequence: Synthetic peptide"
ARDLGTGGMDV

SEQ ID NO: 29 - DNA, 33 bp, Artificial Sequence
  source: /note="Description of Artificial Sequence: Synthetic oligonucleotide"
gcgagagatctgggtacaggaggtatggacgtc

SEQ ID NO: 30 - protein, 107 aa, Artificial Sequence
  source: /note="Description of Artificial Sequence: Synthetic polypeptide"
DIQLTQSPSFLSASVGDRVTITCWASQGISSYLAWYQQKPGKAPKLLIYAASTLQSGVPSRFSGSGSGTEFTLTISSLQPEDFATYYCQQLNSYPLTFGGGTKVEIK

SEQ ID NO: 31 - DNA, 321 bp, Artificial Sequence
  source: /note="Description of Artificial Sequence: Synthetic polynucleotide"
gacatccagttgacccagtctccatccttcctgtctgcatctgtaggagacagagtcaccatcacttgctgggccagtcagggcattagcagttatttagcctggtatcagcaaaaaccagggaaagcccctaagctcctgatctatgctgcatccactttgcaaagtggggtcccatcaaggttcagcggcagtggatctgggacagaattcactctcacaatcagcagcctgcagcctgaagattttgcaacttattactgtcaacagcttaatagttaccctctcactttcggcggagggaccaaggtggagatcaaa

SEQ ID NO: 32 - protein, 6 aa, Artificial Sequence
  source: /note="Description of Artificial Sequence: Synthetic peptide"
QGISSY

SEQ ID NO: 33 - DNA, 18 bp, Artificial Sequence
  source: /note="Description of Artificial Sequence: Synthetic oligonucleotide"
cagggcattagcagttat

SEQ ID NO: 34 - protein, 3 aa, Artificial Sequence
  source: /note="Description of Artificial Sequence: Synthetic peptide"
AAS

SEQ ID NO: 35 - DNA, 9 bp, Artificial Sequence
  source: /note="Description of Artificial Sequence: Synthetic oligonucleotide"
gctgcatcc

SEQ ID NO: 36 - protein, 9 aa, Artificial Sequence
  source: /note="Description of Artificial Sequence: Synthetic peptide"
QQLNSYPLT

SEQ ID NO: 37 - DNA, 27 bp, Artificial Sequence
  source: /note="Description of Artificial Sequence: Synthetic oligonucleotide"
caacagcttaatagttaccctctcact

SEQ ID NO: 38 - protein, 447 aa, Artificial Sequence
  source: /note="Description of Artificial Sequence: Synthetic polypeptide"
EVQLVESGGGLVQPGGSLRLSCAASGLIVSRNYMIWVRQAPGKGLEWVSVIYSGGSTFYADSVKGRFTISRHNSKNTLYLQMNSLRAEDTAVYYCARDLGTGGMDVWGQGTTVTVSSASTKGPSVFPLAPSSKSTSGGTAALGCLVKDYFPEPVTVSWNSGALTSGVHTFPAVLQSSGLYSLSSVVTVPSSSLGTQTYICNVNHKPSNTKVDKKVEPKSCDKTHTCPPCPAPELLGGPSVFLFPPKPKDTLMISRTPEVTCVVVDVSHEDPEVKFNWYVDGVEVHNAKTKPREEQYNSTYRVVSVLTVLHQDWLNGKEYKCKVSNKALPAPIEKTISKAKGQPREPQVYTLPPSRDELTKNQVSLTCLVKGFYPSDIAVEWESNGQPENNYKTTPPVLDSDGSFFLYSKLTVDKSRWQQGNVFSCSVMHEALHNHYTQKSLSLSPGK

SEQ ID NO: 39 - DNA, 1344 bp, Artificial Sequence
  source: /note="Description of Artificial Sequence: Synthetic polynucleotide"
gaggtgcagctggtggagtctggaggaggcttggtccagcctggggggtccctgagactctcctgtgcagcctctgggttaatagtcagtcgcaactacatgatctgggtccgccaggctccagggaaggggctggagtgggtctcagttatttatagcggtggtagcacattctacgcagactccgtgaagggccgattcaccatctccagacacaattccaagaacacgctgtatcttcaaatgaacagcctgagggctgaggacacggccgtatattactgtgcgagagatctgggtacaggaggtatggacgtctggggccaagggaccacggtcaccgtctcctcagcctccaccaagggcccatcggtcttccccctggcaccctcctccaagagcacctctgggggcacagcggccctgggctgcctggtcaaggactacttccccgaaccggtgacggtgtcgtggaactcaggcgccctgaccagcggcgtgcacaccttcccggctgtcctacagtcctcaggactctactccctcagcagcgtggtgaccgtgccctccagcagcttgggcacccagacctacatctgcaacgtgaatcacaagcccagcaacaccaaggtggacaagaaagttgagcccaaatcttgtgacaaaactcacacatgcccaccgtgcccagcacctgaactcctggggggaccgtcagtcttcctcttccccccaaaacccaaggacaccctcatgatctcccggacccctgaggtcacatgcgtggtggtggacgtgagccacgaagaccctgaggtcaagttcaactggtacgtggacggcgtggaggtgcataatgccaagacaaagccgcgggaggagcagtacaacagcacgtaccgtgtggtcagcgtcctcaccgtcctgcaccaggactggctgaatggcaaggagtacaagtgcaaggtctccaacaaagccctcccagcccccatcgagaaaaccatctccaaagccaaagggcagccccgagaaccacaggtgtacaccctgcccccatcccgggatgagctgaccaagaaccaggtcagcctgacctgcctggtcaaaggcttctatcccagcgacatcgccgtggagtgggagagcaatgggcagccggagaacaactacaagaccacgcctcccgtgctggactccgacggctccttcttcctctacagcaagctcaccgtggacaagagcaggtggcagcaggggaacgtcttctcatgctccgtgatgcatgaggctctgcacaaccactacacgcagaagtccctctccctgtctccgggtaaatga

SEQ ID NO: 40 - protein, 214 aa, Artificial Sequence
  source: /note="Description of Artificial Sequence: Synthetic polypeptide"
DIQLTQSPSFLSASVGDRVTITCWASQGISSYLAWYQQKPGKAPKLLIYAASTLQSGVPSRFSGSGSGTEFTLTISSLQPEDFATYYCQQLNSYPLTFGGGTKVEIKRTVAAPSVFIFPPSDEQLKSGTASVVCLLNNFYPREAKVQWKVDNALQSGNSQESVTEQDSKDSTYSLSSTLTLSKADYEKHKVYACEVTHQGLSSPVTKSFNRGEC

SEQ ID NO: 41 - DNA, 645 bp, Artificial Sequence
  source: /note="Description of Artificial Sequence: Synthetic polynucleotide"
gacatccagttgacccagtctccatccttcctgtctgcatctgtaggagacagagtcaccatcacttgctgggccagtcagggcattagcagttatttagcctggtatcagcaaaaaccagggaaagcccctaagctcctgatctatgctgcatccactttgcaaagtggggtcccatcaaggttcagcggcagtggatctgggacagaattcactctcacaatcagcagcctgcagcctgaagattttgcaacttattactgtcaacagcttaatagttaccctctcactttcggcggagggaccaaggtggagatcaaacgaactgtggctgcaccatctgtcttcatcttcccgccatctgatgagcagttgaaatctggaactgcctctgttgtgtgcctgctgaataacttctatcccagagaggccaaagtacagtggaaggtggataacgccctccaatcgggtaactcccaggagagtgtcacagagcaggacagcaaggacagcacctacagcctcagcagcaccctgacgctgagcaaagcagactacgagaaacacaaagtctacgcctgcgaagtcacccatcagggcctgagctcgcccgtcacaaagagcttcaacaggggagagtgttag

SEQ ID NO: 42 - protein, 1254 aa, Artificial Sequence
  source: /note="Description of Artificial Sequence: Synthetic polypeptide"
MFVFLVLLPLVSSQCVNLTTRTQLPPAYTNSFTRGVYYPDKVFRSSVLHSTQDLFLPFFSNVTWFHAIHVSGTNGTKRFDNPVLPFNDGVYFASTEKSNIIRGWIFGTTLDSKTQSLLIVNNATNVVIKVCEFQFCNDPFLGVYYHKNNKSWMESEFRVYSSANNCTFEYVSQPFLMDLEGKQGNFKNLREFVFKNIDGYFKIYSKHTPINLVRDLPQGFSALEPLVDLPIGINITRFQTLLALHRRYLTPGDSSSGWTAGAAAYYVGYLQPRTFLLKYNENGTITDAVDCALDPLSETKCTLKSFTVEKGIYQTSNFRVQPTESIVRFPNITNLCPFGEVFNATRFASVYAWNRKRISNCVADYSVLYNSASFSTFKCYGVSPTKLNDLCFTNVYADSFVIRGDEVRQIAPGQTGKIADYNYKLPDDFTGCVIAWNSNNLDSKVGGNYNYLYRLFRKSNLKPFERDISTEIYQAGSTPCNGVEGFNCYFPLQSYGFQPTNGVGYQPYRVVVLSFELLHAPATVCGPKKSTNLVKNKCVNFNFNGLTGTGVLTESNKKFLPFQQFGRDIADTTDAVRDPQTLEILDITPCSFGGVSVITPGTNTSNQVAVLYQNVNCTEVPVAIHADQLTPTWRVYSTGSNVFQTRAGCLIGAEHVNNSYECDIPIGAGICASYQTQTNSPRRAQSVASQSIIAYTMSLGAENSVAYSNNSIAIPTNFTISVTTEILPVSMTKTSVDCTMYICGDSTECSNLLLQYGSFCTQLNRALTGIAVEQDKNTQEVFAQVKQIYKTPPIKDFGGFNFSQILPDPSKPSKRSFIEDLLFNKVTLADAGFIKQYGDCLGDIAARDLICAQKFNGLTVLPPLLTDEMIAQYTSALLAGTITSGWTFGAGAALQIPFAMQMAYRFNGIGVTQNVLYENQKLIANQFNSAIGKIQDSLSSTASALGKLQDVVNQNAQALNTLVKQLSSNFGAISSVLNDILSRLDKVEAEVQIDRLITGRLQSLQTYVTQQLIRAAEIRASANLAATKMSECVLGQSKRVDFCGKGYHLMSFPQSAPHGVVFLHVTYVPAQEKNFTTAPAICHDGKAHFPREGVFVSNGTHWFVTQRNFYEPQIITTDNTFVSGNCDVVIGIVNNTVYDPLQPELDSFKEELDKYFKNHTSPDVDLGDISGINASVVNIQKEIDRLNEVAKNLNESLIDLQELGKYEQYIKWPWYIWLGFIAGLIAIVMVTIMLCCMTSCCSCLKGCCSCGSCC

SEQ ID NO: 43 - DNA, 3765 bp, Artificial Sequence
  source: /note="Description of Artificial Sequence: Synthetic polynucleotide"
atgttcgtcttcctggtcctgctgcctctggtctcctcacagtgcgtcaatctgacaactcggactcagctgccacctgcttatactaatagcttcaccagaggcgtgtactatcctgacaaggtgtttagaagctccgtgctgcactctacacaggatctgtttctgccattctttagcaacgtgacctggttccacgccatccacgtgagcggcaccaatggcacaaagcggttcgacaatcccgtgctgccttttaacgatggcgtgtacttcgcctctaccgagaagagcaacattatcagaggctggatctttggcaccacactggactccaagacacagtctctgctgatcgtgaacaatgccaccaacgtggtcatcaaggtgtgcgagttccagttttgtaatgatcccttcctgggcgtgtactatcacaagaacaataagagctggatggagtccgagtttagagtgtattctagcgccaacaactgcacatttgagtacgtgagccagcctttcctgatggacctggagggcaagcagggcaatttcaagaacctgagggagttcgtgtttaagaatatcgacggctacttcaaaatctactctaagcacacccccatcaacctggtgcgcgacctgcctcagggcttcagcgccctggagcccctggtggatctgcctatcggcatcaacatcacccggtttcagacactgctggccctgcacagaagatacctgacacccggcgactcctctagcggatggaccgccggcgctgccgcctactatgtgggctacctccagccccggaccttcctgctgaagtacaacgagaatggcaccatcacagacgcagtggattgcgccctggaccccctgagcgagacaaagtgtacactgaagtcctttaccgtggagaagggcatctatcagacatccaatttcagggtgcagccaaccgagtctatcgtgcgctttcctaatatcacaaacctgtgcccatttggcgaggtgttcaacgcaacccgcttcgccagcgtgtacgcctggaataggaagcggatcagcaactgcgtggccgactatagcgtgctgtacaactccgcctctttcagcacctttaagtgctatggcgtgtcccccacaaagctgaatgacctgtgctttaccaacgtctacgccgattctttcgtgatcaggggcgacgaggtgcgccagatcgcccccggccagacaggcaagatcgcagactacaattataagctgccagacgatttcaccggctgcgtgatcgcctggaacagcaacaatctggattccaaagtgggcggcaactacaattatctgtaccggctgtttagaaagagcaatctgaagcccttcgagagggacatctctacagaaatctaccaggccggcagcaccccttgcaatggcgtggagggctttaactgttatttcccactccagtcctacggcttccagcccacaaacggcgtgggctatcagccttaccgcgtggtggtgctgagctttgagctgctgcacgccccagcaacagtgtgcggccccaagaagtccaccaatctggtgaagaacaagtgcgtgaacttcaacttcaacggcctgaccggcacaggcgtgctgaccgagtccaacaagaagttcctgccatttcagcagttcggcagggacatcgcagataccacagacgccgtgcgcgacccacagaccctggagatcctggacatcacaccctgctctttcggcggcgtgagcgtgatcacacccggcaccaatacaagcaaccaggtggccgtgctgtatcagaacgtgaattgtaccgaggtgcccgtggctatccacgccgatcagctgaccccaacatggcgggtgtacagcaccggctccaacgtcttccagacaagagccggatgcctgatcggagcagagcacgtgaacaattcctatgagtgcgacatcccaatcggcgccggcatctgtgcctcttaccagacccagacaaactctcccagaagagcccagagcgtggcctcccagtctatcatcgcctataccatgtccctgggcgccgagaacagcgtggcctactctaacaatagcatcgccatcccaaccaacttcacaatctctgtgaccacagagatcctgcccgtgtccatgaccaagacatctgtggactgcacaatgtatatctgtggcgattctaccgagtgcagcaacctgctgctccagtacggcagcttttgtacccagctgaatagagccctgacaggcatcgccgtggagcaggataagaacacacaggaggtgttcgcccaggtgaagcaaatctacaagaccccccctatcaaggactttggcggcttcaatttttcccagatcctgcctgatccatccaagccttctaagcggagctttatcgaggacctgctgttcaacaaggtgaccctggccgatgccggcttcatcaagcagtatggcgattgcctgggcgacatcgcagccagggacctgatctgcgcccagaagtttaatggcctgaccgtgctgccacccctgctgacagatgagatgatcgcacagtacacaagcgccctgctggccggcaccatcacatccggatggaccttcggcgcaggagccgccctccagatcccctttgccatgcagatggcctataggttcaacggcatcggcgtgacccagaatgtgctgtacgagaaccagaagctgatcgccaatcagtttaactccgccatcggcaagatccaggacagcctgtcctctacagccagcgccctgggcaagctccaggatgtggtgaatcagaacgcccaggccctgaataccctggtgaagcagctgagcagcaacttcggcgccatctctagcgtgctgaatgacatcctgagccggctggacaaggtggaggcagaggtgcagatcgaccggctgatcaccggccggctccagagcctccagacctatgtgacacagcagctgatcagggccgccgagatcagggccagcgccaatctggcagcaaccaagatgtccgagtgcgtgctgggccagtctaagagagtggacttttgtggcaagggctatcacctgatgtccttccctcagtctgccccacacggcgtggtgtttctgcacgtgacctacgtgcccgcccaggagaagaacttcaccacagcccctgccatctgccacgatggcaaggcccactttccaagggagggcgtgttcgtgtccaacggcacccactggtttgtgacacagcgcaatttctacgagccccagatcatcaccacagacaacaccttcgtgagcggcaactgtgacgtggtcatcggcatcgtgaacaataccgtgtatgatccactccagcccgagctggacagctttaaggaggagctggataagtatttcaagaatcacacctcccctgacgtggatctgggcgacatcagcggcatcaatgcctccgtggtgaacatccagaaggagatcgaccgcctgaacgaggtggctaagaatctgaacgagagcctgatcgacctccaggagctgggcaagtatgagcagtacatcaagtggccctggtacatctggctgggcttcatcgccggcctgatcgccatcgtgatggtgaccatcatgctgtgctgtatgacatcctgctgttcttgcctgaagggctgctgtagctgtggctcctgctgttaa

SEQ ID NO: 44 - protein, 1252 aa, Artificial Sequence
  source: /note="Description of Artificial Sequence: Synthetic polypeptide"
MFVFLVLLPLVSSQCVNLTTRTQLPPAYTNSFTRGVYYPDKVFRSSVLHSTQDLFLPFFSNVTWFHAISGTNGTKRFDNPVLPFNDGVYFASTEKSNIIRGWIFGTTLDSKTQSLLIVNNATNVVIKVCEFQFCNDPFLGVYYHKNNKSWMESEFRVYSSANNCTFEYVSQPFLMDLEGKQGNFKNLREFVFKNIDGYFKIYSKHTPINLVRDLPQGFSALEPLVDLPIGINITRFQTLLALHRSYLTPGDSSSGWTAGAAAYYVGYLQPRTFLLKYNENGTITDAVDCALDPLSETKCTLKSFTVEKGIYQTSNFRVQPTESIVRFPNITNLCPFGEVFNATRFASVYAWNRKRISNCVADYSVLYNSASFSTFKCYGVSPTKLNDLCFTNVYADSFVIRGDEVRQIAPGQTGKIADYNYKLPDDFTGCVIAWNSNNLDSKVGGNYNYLYRLFRKSNLKPFERDISTEIYQAGSTPCNGVKGFNCYFPLQSYGFQPTYGVGYQPYRVVVLSFELLHAPATVCGPKKSTNLVKNKCVNFNFNGLTGTGVLTESNKKFLPFQQFGRDIADTTDAVRDPQTLEILDITPCSFGGVSVITPGTNTSNQVAVLYQGVNCTEVPVAIHADQLTPTWRVYSTGSNVFQTRAGCLIGAEHVNNSYECDIPIGAGICASYQTQTNSPRRARSVASQSIIAYTMSLGAENSVAYSNNSIAIPTNFTISVTTEILPVSMTKTSVDCTMYICGDSTECSNLLLQYGSFCTQLNRALTGIAVEQDKNTQEVFAQVKQIYKTPPIKDFGGFNFSQILPDPSKPSKRSFIEDLLFNKVTLADAGFIKQYGDCLGDIAARDLICAQKFNGLTVLPPLLTDEMIAQYTSALLAGTITSGWTFGAGAALQIPFAMQMAYRFNGIGVTQNVLYENQKLIANQFNSAIGKIQDSLSSTASALGKLQDVVNQNAQALNTLVKQLSSNFGAISSVLNDILSRLDKVEAEVQIDRLITGRLQSLQTYVTQQLIRAAEIRASANLAATKMSECVLGQSKRVDFCGKGYHLMSFPQSAPHGVVFLHVTYVPAQEKNFTTAPAICHDGKAHFPREGVFVSNGTHWFVTQRNFYEPQIITTDNTFVSGNCDVVIGIVNNTVYDPLQPELDSFKEELDKYFKNHTSPDVDLGDISGINASVVNIQKEIDRLNEVAKNLNESLIDLQELGKYEQYIKWPWYIWLGFIAGLIAIVMVTIMLCCMTSCCSCLKGCCSCGSCC

SEQ ID NO: 45 - protein, 119 aa, Artificial Sequence
  source: /note="Description of Artificial Sequence: Synthetic polypeptide"
EVQLVESGGGLVQPGGSLRLSCAASGFTFSIYEMNWVRQAPGKGLEWVSYITSSGTTIYYADSVKGRFTISRDNAKNSLYLQMNSLRAEDTAVYYCASSSSSGYYFDYWGQGTLVTVSS

SEQ ID NO: 46 - protein, 8 aa, Artificial Sequence
  source: /note="Description of Artificial Sequence: Synthetic peptide"
GFTFSIYE

SEQ ID NO: 47 - protein, 8 aa, Artificial Sequence
  source: /note="Description of Artificial Sequence: Synthetic peptide"
ITSSGTTI

SEQ ID NO: 48 - protein, 12 aa, Artificial Sequence
  source: /note="Description of Artificial Sequence: Synthetic peptide"
ASSSSSGYYFDY

SEQ ID NO: 49 - protein, 113 aa, Artificial Sequence
  source: /note="Description of Artificial Sequence: Synthetic polypeptide"
DIVMTQSPDSLAVSLGERATINCKSSQSVLYSSNNKNYLAWYQQKPGQPPNLLIYWASTRESGVPDRFSGSGSGTDFTLTISSLQAEDVAVYYCQQYYSTPPTFGQGTKLEIK

SEQ ID NO: 50 - protein, 12 aa, Artificial Sequence
  source: /note="Description of Artificial Sequence: Synthetic peptide"
QSVLYSSNNKNY

SEQ ID NO: 51 - protein, 3 aa, Artificial Sequence
  source: /note="Description of Artificial Sequence: Synthetic peptide"
WAS

SEQ ID NO: 52 - protein, 9 aa, Artificial Sequence
  source: /note="Description of Artificial Sequence: Synthetic peptide"
QQYYSTPPT

SEQ ID NO: 53 - protein, 449 aa, Artificial Sequence
  source: /note="Description of Artificial Sequence: Synthetic polypeptide"
EVQLVESGGGLVQPGGSLRLSCAASGFTFSIYEMNWVRQAPGKGLEWVSYITSSGTTIYYADSVKGRFTISRDNAKNSLYLQMNSLRAEDTAVYYCASSSSSGYYFDYWGQGTLVTVSSASTKGPSVFPLAPSSKSTSGGTAALGCLVKDYFPEPVTVSWNSGALTSGVHTFPAVLQSSGLYSLSSVVTVPSSSLGTQTYICNVNHKPSNTKVDKKVEPKSCDKTHTCPPCPAPELLGGPSVFLFPPKPKDTLMISRTPEVTCVVVDVSHEDPEVKFNWYVDGVEVHNAKTKPREEQYNSTYRVVSVLTVLHQDWLNGKEYKCKVSNKALPAPIEKTISKAKGQPREPQVYTLPPSRDELTKNQVSLTCLVKGFYPSDIAVEWESNGQPENNYKTTPPVLDSDGSFFLYSKLTVDKSRWQQGNVFSCSVMHEALHNHYTQKSLSLSPGK

SEQ ID NO: 54 - protein, 220 aa, Artificial Sequence
  source: /note="Description of Artificial Sequence: Synthetic polypeptide"
DIVMTQSPDSLAVSLGERATINCKSSQSVLYSSNNKNYLAWYQQKPGQPPNLLIYWASTRESGVPDRFSGSGSGTDFTLTISSLQAEDVAVYYCQQYYSTPPTFGQGTKLEIKRTVAAPSVFIFPPSDEQLKSGTASVVCLLNNFYPREAKVQWKVDNALQSGNSQESVTEQDSKDSTYSLSSTLTLSKADYEKHKVYACEVTHQGLSSPVTKSFNRGEC

SEQ ID NO: 55 - DNA, 357 bp, Artificial Sequence
  source: /note="Description of Artificial Sequence: Synthetic polynucleotide"
gaggtgcagctggtggagtctgggggaggcttggtacagcctggagggtccctgagactctcctgtgcagcctctggattcaccttcagtatttatgaaatgaactgggtccgccaggctccagggaaggggctggagtgggtttcatacattactagtagtggtactaccatatactacgcagactctgtgaagggccgattcaccatctccagagacaacgccaagaactcactgtatctgcaaatgaacagcctgagagccgaggacacggctgtttattactgtgcgagtagcagctcgtccgggtactactttgactactggggccagggaaccctggtcaccgtctcctca

SEQ ID NO: 56 - DNA, 24 bp, Artificial Sequence
  source: /note="Description of Artificial Sequence: Synthetic oligonucleotide"
ggattcaccttcagtatttatgaa

SEQ ID NO: 57 - DNA, 24 bp, Artificial Sequence
  source: /note="Description of Artificial Sequence: Synthetic oligonucleotide"
attactagtagtggtactaccata

SEQ ID NO: 58 - DNA, 36 bp, Artificial Sequence
  source: /note="Description of Artificial Sequence: Synthetic oligonucleotide"
gcgagtagcagctcgtccgggtactactttgactac

SEQ ID NO: 59 - DNA, 339 bp, Artificial Sequence
  source: /note="Description of Artificial Sequence: Synthetic polynucleotide"
gacatcgtgatgacccagtctccagactccctggctgtgtctctgggcgagagggccaccatcaactgcaagtccagccagagtgttttatacagctccaacaataagaactacttagcttggtaccagcagaaaccaggacagcctcctaatctgctcatttactgggcatctacccgggaatccggggtccctgaccgattcagtggcagcgggtctgggacagatttcactctcaccatcagcagcctgcaggctgaagatgtggcagtttattactgtcagcaatattatagtactcctcccacttttggccaggggaccaagctggagatcaaa

SEQ ID NO: 60 - DNA, 36 bp, Artificial Sequence
  source: /note="Description of Artificial Sequence: Synthetic oligonucleotide"
cagagtgttttatacagctccaacaataagaactac

SEQ ID NO: 61 - DNA, 9 bp, Artificial Sequence
  source: /note="Description of Artificial Sequence: Synthetic oligonucleotide"
tgggcatct

SEQ ID NO: 62 - DNA, 27 bp, Artificial Sequence
  source: /note="Description of Artificial Sequence: Synthetic oligonucleotide"
cagcaatattatagtactcctcccact

SEQ ID NO: 63 - DNA, 1350 bp, Artificial Sequence
  source: /note="Description of Artificial Sequence: Synthetic polynucleotide"
gaggtgcagctggtggagtctgggggaggcttggtacagcctggagggtccctgagactctcctgtgcagcctctggattcaccttcagtatttatgaaatgaactgggtccgccaggctccagggaaggggctggagtgggtttcatacattactagtagtggtactaccatatactacgcagactctgtgaagggccgattcaccatctccagagacaacgccaagaactcactgtatctgcaaatgaacagcctgagagccgaggacacggctgtttattactgtgcgagtagcagctcgtccgggtactactttgactactggggccagggaaccctggtcaccgtctcctcagcctccaccaagggcccatcggtcttccccctggcaccctcctccaagagcacctctgggggcacagcggccctgggctgcctggtcaaggactacttccccgaaccggtgacggtgtcgtggaactcaggcgccctgaccagcggcgtgcacaccttcccggctgtcctacagtcctcaggactctactccctcagcagcgtggtgaccgtgccctccagcagcttgggcacccagacctacatctgcaacgtgaatcacaagcccagcaacaccaaggtggacaagaaagttgagcccaaatcttgtgacaaaactcacacatgcccaccgtgcccagcacctgaactcctggggggaccgtcagtcttcctcttccccccaaaacccaaggacaccctcatgatctcccggacccctgaggtcacatgcgtggtggtggacgtgagccacgaagaccctgaggtcaagttcaactggtacgtggacggcgtggaggtgcataatgccaagacaaagccgcgggaggagcagtacaacagcacgtaccgtgtggtcagcgtcctcaccgtcctgcaccaggactggctgaatggcaaggagtacaagtgcaaggtctccaacaaagccctcccagcccccatcgagaaaaccatctccaaagccaaagggcagccccgagaaccacaggtgtacaccctgcccccatcccgggatgagctgaccaagaaccaggtcagcctgacctgcctggtcaaaggcttctatcccagcgacatcgccgtggagtgggagagcaatgggcagccggagaacaactacaagaccacgcctcccgtgctggactccgacggctccttcttcctctacagcaagctcaccgtggacaagagcaggtggcagcaggggaacgtcttctcatgctccgtgatgcatgaggctctgcacaaccactacacgcagaagtccctctccctgtctccgggtaaatga

SEQ ID NO: 64 - DNA, 663 bp, Artificial Sequence
  source: /note="Description of Artificial Sequence: Synthetic polynucleotide"
gacatcgtgatgacccagtctccagactccctggctgtgtctctgggcgagagggccaccatcaactgcaagtccagccagagtgttttatacagctccaacaataagaactacttagcttggtaccagcagaaaccaggacagcctcctaatctgctcatttactgggcatctacccgggaatccggggtccctgaccgattcagtggcagcgggtctgggacagatttcactctcaccatcagcagcctgcaggctgaagatgtggcagtttattactgtcagcaatattatagtactcctcccacttttggccaggggaccaagctggagatcaaacgaactgtggctgcaccatctgtcttcatcttcccgccatctgatgagcagttgaaatctggaactgcctctgttgtgtgcctgctgaataacttctatcccagagaggccaaagtacagtggaaggtggataacgccctccaatcgggtaactcccaggagagtgtcacagagcaggacagcaaggacagcacctacagcctcagcagcaccctgacgctgagcaaagcagactacgagaaacacaaagtctacgcctgcgaagtcacccatcagggcctgagctcgcccgtcacaaagagcttcaacaggggagagtgttag

SEQ ID NO: 65 - protein, 11 aa, Severe acute respiratory syndrome coronavirus 2
QTNSPRRARSV

SEQ ID NO: 66 - protein, 7 aa, Artificial Sequence
  source: /note="Description of Artificial Sequence: Synthetic peptide"
QTILRSV

SEQ ID NO: 67 - protein, 11 aa, Artificial Sequence
  source: /note="Description of Artificial Sequence: Synthetic peptide"
QTNSPGSASSV

SEQ ID NO: 68 - protein, 4 aa, Vesicular stomatitis virus
PPPY

SEQ ID NO: 69 - protein, 4 aa, Artificial Sequence
  source: /note="Description of Artificial Sequence: Synthetic peptide"
APPY

SEQ ID NO: 70 - protein, 4 aa, Artificial Sequence
  source: /note="Description of Artificial Sequence: Synthetic peptide"
AAPY

SEQ ID NO: 71 - protein, 4 aa, Artificial Sequence
  source: /note="Description of Artificial Sequence: Synthetic peptide"
PPAY

SEQ ID NO: 72 - protein, 4 aa, Artificial Sequence
  source: /note="Description of Artificial Sequence: Synthetic peptide"
APPA

SEQ ID NO: 73 - protein, 4 aa, Artificial Sequence
  source: /note="Description of Artificial Sequence: Synthetic peptide"
AAPA

SEQ ID NO: 74 - protein, 4 aa, Artificial Sequence
  source: /note="Description of Artificial Sequence: Synthetic peptide"
PPPA

SEQ ID NO: 75 - protein, 4 aa, Vesicular stomatitis virus
PSAP